European Patent Specification EP 3 325 662 B1, published August 30, 2023. Title: EPIGENETIC SILENCING OF NMT2. Applicant: Pacylex pharmaceuticals Inc. Berthiaume, Luc Beauchamp, Erwan. The sequence listing filed with the application follows.

SEQUENCE LISTING (8 sequences)

SEQ ID NO: 1 - DNA, 25 bp, Artificial Sequence
  Primer
gttttgttttttgttttgttgagat

SEQ ID NO: 2 - DNA, 26 bp, Artificial Sequence
  Primer
tccttttatattttaaccccatttac

SEQ ID NO: 3 - DNA, 26 bp, Artificial Sequence
  Primer
tttaataaggatggtagggagtagag

SEQ ID NO: 4 - DNA, 25 bp, Artificial Sequence
  Primer
accaaccaacaaaacctaaaactaa

SEQ ID NO: 5 - DNA, 26 bp, Artificial Sequence
  Primer
gatttaataaggatggtagggagtag

SEQ ID NO: 6 - DNA, 23 bp, Artificial Sequence
  Primer
actcccaaaactaaaaattcttc

SEQ ID NO: 7 - DNA, 24 bp, Artificial Sequence
  Primer
ggttttgttttgaagagttttagg

SEQ ID NO: 8 - DNA, 25 bp, Artificial Sequence
  Primer
actccctaccatccttattaaatcc